European Patent Application EP 4 212 546 A1, published July 19, 2023. Title: METHODS OF PRODUCING LONG ACTING CTP-MODIFIED POLYPEPTIDES. Applicant: Opko Biologics Ltd. The sequence listing filed with the application follows.

SEQUENCE LISTING (115 sequences)

SEQ ID NO: 1 - protein, 220 aa, Artificial Sequence
  CTP-modified EPO
MGVHECPAWLWLLLSLLSLPLGLPVLGAPPRLICDSRVLERYLLEAKEAENITTGCAEHCSLNENITVPDTVNFYAWKRMEVGQQAVEVWQGLALLSEAVLRGQALLVNSSQPWEPLQLHVDKAVSGLRSLTTLLRALGAQKEAISPPDAASAAPLRTITADTFRKLFRVYSNFLRGKLKLYTGEACRTGDRSSSSKAPPPSLPSPSRLPGPSDTPILPQ

SEQ ID NO: 2 - protein, 248 aa, Artificial Sequence
  CTP-modified EPO
MGVHECPAWLWLLLSLLSLPLGLPVLGAPPRLICDSRVLERYLLEAKEAENITTGCAEHCSLNENITVPDTVNFYAWKRMEVGQQAVEVWQGLALLSEAVLRGQALLVNSSQPWEPLQLHVDKAVSGLRSLTTLLRALGAQKEAISPPDAASAAPLRTITADTFRKLFRVYSNFLRGKLKLYTGEACRTGDRSSSSKAPPPSLPSPSRLPGPSDTPILPQSSSSKAPPPSLPSPSRLPGPSDTPILPQ

SEQ ID NO: 3 - protein, 277 aa, Artificial Sequence
  CTP-modified EPO
MGVHECPAWLWLLLSLLSLPLGLPVLGSSSSKAPPPSLPSPSRLPGPSDTPILPQAPPRLICDSRVLERYLLEAKEAENITTGCAEHCSLNENITVPDTKVNFYAWKRMEVGQQAVEVWQGLALLSEAVLRGQALLVNSSQPWEPLQLHVDKAVSGLRSLTTLLRALGAQKEAISPPDAASAAPLRTITADTFRKLFRVYSNFLRGKLKLYTGEACRTGDRSSSSKAPPPSLPSPSRLPGPSDTPILPQSSSSKAPPPSLPSPSRLPGPSDTPILPQ

SEQ ID NO: 4 - protein, 387 aa, Artificial Sequence
  CTP-modified EPO
MGVHECPAWLWLLLSLLSLPLGLPVLGAPPRLICDSRVLERYLLEAKEAENITTGCAEHCSLNENITVPDTKVNFYAWKRMEVGQQAVEVWQGLALLSEAVLRGQALLVNSSQPWEPLQLHVDKAVSGLRSLTTLLRALGAQKEAISPPDAASAAPLRTITADTFRKLFRVYSNFLRGKLKLYTGEACRTGDRSSSSKAPPPSLPSPSRLPGPSDTPILPQAPPRLICDSRVLERYLLEAKEAENITTGCAEHCSLNENITVPDTKVNFYAWKRMEVGQQAVEVWQGLALLSEAVLRGQALLVNSSQPWEPLQLHVDKAVSGLRSLTTLLRALGAQKEAISPPDAASAAPLRTITADTFRKLFRVYSNFLRGKLKLYTGEACRTGDR

SEQ ID NO: 5 - protein, 221 aa, Artificial Sequence
  CTP-modified EPO
MGVHECPAWLWLLLSLLSLPLGLPVLGSSSSKAPPPSLPSPSRLPGPSDTPILPQAPPRLICDSRVLERYLLEAKEAENITTGCAEHCSLNENITVPDTKVNFYAWKRMEVGQQAVEVWQGLALLSEAVLRGQALLVNSSQPWEPLQLHVDKAVSGLRSLTTLLRALGAQKEAISPPDAASAAPLRTITADTFRKLFRVYSNFLRGKLKLYTGEACRTGDR

SEQ ID NO: 6 - protein, 249 aa, Artificial Sequence
  CTP-modified EPO
MGVHECPAWLWLLLSLLSLPLGLPVLGSSSSKAPPPSLPSPSRLPGPSDTPILPQAPPRLICDSRVLERYLLEAKEAENITTGCAEHCSLNENITVPDTKVNFYAWKRMEVGQQAVEVWQGLALLSEAVLRGQALLVNSSQPWEPLQLHVDKAVSGLRSLTTLLRALGAQKEAISPPDAASAAPLRTITADTFRKLFRVYSNFLRGKLKLYTGEACRTGDRSSSSKAPPPSLPSPSRLPGPSDTPILPQ

SEQ ID NO: 7 - protein, 220 aa, Artificial Sequence
  CTP-modified EPO
MGVHECPAWLWLLLSLLSLPLGLPVLGAPPRLICDSRVLERYLLEAKEAENITTGCAEHCSLNENITVPDTVNFYAWKRMEVGQQAVEVWQGLALLSEAVLRSQALLVNSSQPWEPLQLHVDKAVSGLRSLTTLLRALGAQKEAISPPDAASAAPLRTITADTFRKLFRVYSNFLRGKLKLYTGEACRTGDRSSSSKAPPPSLPSPSRLPGPSDTPILPQ

SEQ ID NO: 8 - protein, 193 aa, Artificial Sequence
  CTP-modified EPO
MGVHECPAWLWLLLSLLSLPLGLPVLGAPPRLICDSRVLERYLLEAKEAENITTGCAEHCSLNENITVPDTKVNFYAWKRMEVGQQAVEVWQGLALLSEAVLRGQALLVNSSQPWEPLQLHVDKAVSGLRSLTTLLRALGAQKEAISPPDAASAAPLRTITADTFRKLFRVYSNFLRGKLKLYTGEACRTGDR

SEQ ID NO: 9 - protein, 271 aa, Artificial Sequence
  CTP-mofied IFN
MTNKCLLQIALLLCFSTTALSSSSSKAPPPSLPSPSRLPGPSDTPILPQMSYNLLGFLQRSSNFQCQKLLWQLNGRLEYCLKDRMNFDIPEEIKQLQQFQKEDAALTIYEMLQNIFAIFRQDSSSTGWNETIVENLLANVYHQINHLKTVLEEKLEKEDFTRGKLMSSLHLKRYYGRILHYLKAKEYSHCAWTIVRVEILRNFYFINRLTGYLRNSSSSKAPPPSLPSPSRLPGPSDTPILPQSSSSKAPPPSLPSPSRLPGPSDTPILPQ

SEQ ID NO: 10 - protein, 243 aa, Artificial Sequence
  CTP-modified IFN
MTNKCLLQIALLLCFSTTALSSSSSKAPPPSLPSPSRLPGPSDTPILPQMSYNLLGFLQRSSNFQCQKLLWQLNGRLEYCLKDRMNFDIPEEIKQLQQFQKEDAALTIYEMLQNIFAIFRQDSSSTGWNETIVENLLANVYHQINHLKTVLEEKLEKEDFTRGKLMSSLHLKRYYGRILHYLKAKEYSHCAWTIVRVEILRNFYFINRLTGYLRNSSSSKAPPPSLPSPSRLPGPSDTPILPQ

SEQ ID NO: 11 - protein, 215 aa, Artificial Sequence
  CTP-modified IFN
MTNKCLLQIALLLCFSTTALSSSSSKAPPPSLPSPSRLPGPSDTPILPQMSYNLLGFLQRSSNFQCQKLLWQLNGRLEYCLKDRMNFDIPEEIKQLQQFQKEDAALTIYEMLQNIFAIFRQDSSSTGWNETIVENLLANVYHQINHLKTVLEEKLEKEDFTRGKLMSSLHLKRYYGRILHYLKAKEYSHCAWTIVRVEILRNFYFINRLTGYLRN

SEQ ID NO: 12 - protein, 243 aa, Artificial Sequence
  CTP-modified IFN
MTNKCLLQIALLLCFSTTALSMSYNLLGFLQRSSNFQCQKLLWQLNGRLEYCLKDRMNFDIPEEIKQLQQFQKEDAALTIYEMLQNIFAIFRQDSSSTGWNETIVENLLANVYHQINHLKTVLEEKLEKEDFTRGKLMSSLHLKRYYGRILHYLKAKEYSHCAWTIVRVEILRNFYFINRLTGYLRNSSSSKAPPPSLPSPSRLPGPSDTPILPQSSSSKAPPPSLPSPSRLPGPSDTPILPQ

SEQ ID NO: 13 - protein, 215 aa, Artificial Sequence
  CTP-modified IFN
MTNKCLLQIALLLCFSTTALSMSYNLLGFLQRSSNFQCQKLLWQLNGRLEYCLKDRMNFDIPEEIKQLQQFQKEDAALTIYEMLQNIFAIFRQDSSSTGWNETIVENLLANVYHQINHLKTVLEEKLEKEDFTRGKLMSSLHLKRYYGRILHYLKAKEYSHCAWTIVRVEILRNFYFINRLTGYLRNSSSSKAPPPSLPSPSRLPGPSDTPILPQ

SEQ ID NO: 14 - protein, 32 aa, Artificial Sequence
  CTP-peptide
DPRFQDSSSSKAPPPSLPSPSRLPGPSDTPIL

SEQ ID NO: 15 - protein, 28 aa, Artificial Sequence
  CTP-peptide
SSSSKAPPPSLPSPSRLPGPSDTPILPQ

SEQ ID NO: 16 - protein, 12 aa, Artificial Sequence
  CTP-peptide
SSSSKAPPPSLP

SEQ ID NO: 17 - DNA, 786 bp, Artificial Sequence
  CTP-modified EPO
tctagaggtcatcatgggggtgcacgaatgtcctgcctggctgtggcttctcctgtcccttctgtcgctccctctgggcctcccagtcctgggctcctcttcctcaaaggcccctcccccgagccttccaagtccatcccgactcccggggccctcggacaccccaatattaccacaagccccaccacgcctcatctgtgacagccgagtcctggagaggtacctcttggaggccaaggaggccgagaatatcacgacgggctgtgctgaacactgcagcttgaatgagaatatcactgtcccagacaccaaagttaatttctatgcctggaagaggatggaggtcgggcagcaggccgtagaagtctggcagggcctggccctgctgtcggaagctgtcctgcggggccaggccctgttggtcaactcttcccagccgtgggagcccctgcagctgcatgtggataaagccgtcagtggccttcgcagcctcaccactctgcttcgggctctgggagcccagaaggaagccatctcccctccagatgcggcctcagctgctccactccgaacaatcactgctgacactttccgcaaactcttccgagtctactccaatttcctccggggaaagctgaagctgtacacaggggaggcctgcaggacaggggacagatcctcttcctcaaaggcccctcccccgagccttccaagtccatcccgactcccggggccctcggacaccccgatcctcccacaataaaggtcttctggatccgcggccgc

SEQ ID NO: 18 - DNA, 873 bp, Artificial Sequence
  CTP-modified EPO
tctagaggtcatcatgggggtgcacgaatgtcctgcctggctgtggcttctcctgtcccttctgtcgctccctctgggcctcccagtcctgggctcctcttcctcaaaggcccctcccccgagccttccaagtccatcccgactcccggggccctcggacaccccaatattaccacaagccccaccacgcctcatctgtgacagccgagtcctggagaggtacctcttggaggccaaggaggccgagaatatcacgacgggctgtgctgaacactgcagcttgaatgagaatatcactgtcccagacaccaaagttaatttctatgcctggaagaggatggaggtcgggcagcaggccgtagaagtctggcagggcctggccctgctgtcggaagctgtcctgcggggccaggccctgttggtcaactcttcccagccgtgggagcccctgcagctgcatgtggataaagccgtcagtggccttcgcagcctcaccactctgcttcgggctctgggagcccagaaggaagccatctcccctccagatgcggcctcagctgctccactccgaacaatcactgctgacactttccgcaaactcttccgagtctactccaatttcctccggggaaagctgaagctgtacacaggggaggcctgcaggacaggggacagatcctcttcctcaaaggcccctcccccgagccttccaagtccatcccgactcccggggccctccgacacaccaatcctgccacagagcagctcctctaaggcccctcctccatccctgccatccccctcccggctgcctggcccctctgacacccctatcctgcctcagtgatgaaggtcttctggatccgcggccgc

SEQ ID NO: 19 - protein, 27 aa, Artificial Sequence
  EPO signal peptide
MGVHECPAWLWLLLSLLSLPLGLPVLG

SEQ ID NO: 20 - protein, 166 aa, Artificial Sequence
  IFN-beta
MSYNLLGFLQRSSNFQSQKLLWQLNGRLEYCLKDRMNFDIPEEIKQLQQFQKEDAALTIYEMLQNIFAIFRQDSSSTGWNETIVENLLANVYHQINHLKTVLEEKLEKEDFTRGKLMSSLHLKRYYGRILHYLKAKEYSHCAWTIVRVEILRNFYFINRLTGYLRN

SEQ ID NO: 21 - protein, 30 aa, Artificial Sequence
  GLP-1
HAEGTFTSDVSSYLEGQAAKEFIAWLVKGR

SEQ ID NO: 22 - DNA, 661 bp, Artificial Sequence
  CTP-modified IFN
tctagaggacatgaccaacaagtgcctgctgcagatcgccctgctgctgtgcttcagcaccaccgccctgagcatgagctacaacctgctgggcttcctgcagaggtccagcaacttccagtgccagaagctgctgtggcagctgaacggcaggctggaatactgcctgaaggacaggatgaacttcgacatcccagaggaaatcaagcagctgcagcagttccagaaggaggacgccgccctgaccatctacgagatgctgcagaacatcttcgccatcttcaggcaggacagcagcagcaccggctggaacgagaccatcgtggagaacctgctggccaacgtgtaccaccagatcaaccacctgaaaaccgtgctggaagagaagctggaaaaggaggacttcaccaggggcaagctgatgagcagcctgcacctgaagaggtactacggcagaatcctgcactacctgaaggccaaggagtacagccactgcgcctggaccatcgtgagggtggagatcctgaggaacttctacttcatcaacaggctgaccggctacctgaggaacagctccagcagcaaggcccctccaccttccctgcccagtccaagccgactccctgggccctccgatacaccaattctgccacagtgatga

SEQ ID NO: 23 - DNA, 765 bp, Artificial Sequence
  CTP-modified IFN
tctagaggacatgaccaacaagtgcctgctgcagatcgccctgctgctgtgcttcagcaccaccgccctgagcatgagctacaacctgctgggcttcctgcagaggtccagcaacttccagtgccagaagctgctgtggcagctgaacggcaggctggaatactgcctgaaggacaggatgaacttcgacatcccagaggaaatcaagcagctgcagcagttccagaaggaggacgccgccctgaccatctacgagatgctgcagaacatcttcgccatcttcaggcaggacagcagcagcaccggctggaacgagaccatcgtggagaacctgctggccaacgtgtaccaccagatcaaccacctgaaaaccgtgctggaagagaagctggaaaaggaggacttcaccaggggcaagctgatgagcagcctgcacctgaagaggtactacggcagaatcctgcactacctgaaggccaaggagtacagccactgcgcctggaccatcgtgagggtggagatcctgaggaacttctacttcatcaacaggctgaccggctacctgaggaacagctccagcagcaaggcccctccaccttccctgcccagtccaagccgactccctgggccctccgacacaccaatcctgccacagagcagctcctctaaggcccctcctccatccctgccatccccctcccggctgcctggcccctctgacacccctatcctgcctcagtgatgaaggtctggatccgcggccgc

SEQ ID NO: 24 - DNA, 849 bp, Artificial Sequence
  CTP-modified IFN
tctagaggacatgaccaacaagtgcctgctgcagatcgccctgctgctgtgcttcagcaccaccgccctgagcagcagcagctccaaggccccaccccccagcctgcccagccccagcagactgccaggccccagcgacacccccatcctgccccagatgagctacaacctgctgggcttcctgcagaggtccagcaacttccagtgccagaagctgctgtggcagctgaacggcaggctggaatactgcctgaaggacaggatgaacttcgacatcccagaggaaatcaagcagctgcagcagttccagaaggaggacgccgccctgaccatctacgagatgctgcagaacatcttcgccatcttcaggcaggacagcagcagcaccggctggaacgagaccatcgtggagaacctgctggccaacgtgtaccaccagatcaaccacctgaaaaccgtgctggaagagaagctggaaaaggaggacttcaccaggggcaagctgatgagcagcctgcacctgaagaggtactacggcagaatcctgcactacctgaaggccaaggagtacagccactgcgcctggaccatcgtgagggtggagatcctgaggaacttctacttcatcaacaggctgaccggctacctgaggaacagctccagcagcaaggcccctccaccttccctgcccagtccaagccgactccctgggccctccgacacaccaatcctgccacagagcagctcctctaaggcccctcctccatccctgccatccccctcccggctgcctggcccctctgacacccctatcctgcctcagtgatgaaggtctggatccgcggccgc

SEQ ID NO: 25 - protein, 409 aa, Artificial Sequence
  CTP-modified IFN
MTNKCLLQIALLLCFSTTALSSSSSKAPPPSLPSPSRLPGPSDTPILPQMSYNLLGFLQRSSNFQCQKLLWQLNGRLEYCLKDRMNFDIPEEIKQLQQFQKEDAALTIYEMLQNIFAIFRQDSSSTGWNETIVENLLANVYHQINHLKTVLEEKLEKEDFTRGKLMSSLHLKRYYGRILHYLKAKEYSHCAWTIVRVEILRNFYFINRLTGYLRNSSSSKAPPPSLPSPSRLPGPSDTPILPQMSYNLLGFLQRSSNFQCQKLLWQLNGRLEYCLKDRMNFDIPEEIKQLQQFQKEDAALTIYEMLQNIFAIFRQDSSSTGWNETIVENLLANVYHQINHLKTVLEEKLEKEDFTRGKLMSSLHLKRYYGRILHYLKAKEYSHCAWTIVRVEILRNFYFINRLTGYLRN

SEQ ID NO: 26 - DNA, 1261 bp, Artificial Sequence
  CTP-modified IFN
tctagaggacatgaccaacaagtgcctgctgcagatcgccctgctgctgtgcttcagcaccaccgccctgagcagcagcagctccaaggccccaccccccagcctgcccagccccagcaggctgccaggccccagcgacacccccatcctgccccagatgagctacaacctgctgggcttcctgcagaggtccagcaacttccagtgccagaaactgctgtggcagctgaacggcaggctggaatactgcctgaaggaccggatgaacttcgacatccccgaagagatcaagcagctgcagcagttccagaaagaggacgccgccctgaccatctacgagatgctgcagaacatcttcgccatcttcaggcaggacagcagcagcaccggctggaacgagaccatcgtggagaacctgctggccaacgtgtaccaccagatcaaccacctgaaaaccgtgctggaagagaagctggaaaaagaggacttcaccaggggcaagctgatgagcagcctgcacctgaagaggtactacggcagaatcctgcactacctgaaggccaaagagtacagccactgcgcctggaccatcgtgagggtggagatcctgcggaacttctacttcatcaacaggctgaccggctacctgaggaacagctccagcagcaaggcccctccaccctccctgccctccccaagcagactgcccggaccctccgacacaccaattctgccacagatgtcctacaatctgctcggatttctgcagcgctcctccaactttcagtgtcagaagctcctctggcagctcaatggccgcctggaatattgtctgaaagacagaatgaattttgacatcccagaggaaattaaacagctccagcagtttcagaaagaagatgctgctctcacaatctatgaaatgctccagaatatctttgcaatctttcgccaggacagctcctccaccgggtggaatgagacaattgtcgagaatctgctcgccaatgtctatcatcagatcaatcacctcaagacagtcctcgaagaaaaactcgaaaaagaagatttcacacgcggcaaactgatgtcctccctgcatctgaagcgctactatgggcgcatcctgcattatctgaaagctaaagaatactcccactgtgcttggacaattgtgcgcgtcgagatcctgagaaacttttatttcattaaccgcctgacaggatacctgcgcaactgatgaaggtctggatgcggccgc

SEQ ID NO: 27 - DNA, 673 bp, Artificial Sequence
  CTP-modified IFN
tctagaggacatgaccaacaagtgcctgctgcagatcgccctgctgctgtgcttcagcaccaccgccctgagcagcagcagctccaaggccccaccccccagcctgcccagccccagcaggctgccaggccccagcgacacccccatcctgccccagatgagctacaacctgctgggcttcctgcagaggtccagcaacttccagtgccagaaactgctgtggcagctgaacggcaggctggaatactgcctgaaggaccggatgaacttcgacatccccgaagagatcaagcagctgcagcagttccagaaagaggacgccgccctgaccatctacgagatgctgcagaacatcttcgccatcttcaggcaggacagcagcagcaccggctggaacgagaccatcgtggagaacctgctggccaacgtgtaccaccagatcaaccacctgaaaaccgtgctggaagagaagctggaaaaagaggacttcaccaggggcaagctgatgagcagcctgcacctgaagaggtactacggcagaatcctgcactacctgaaggccaaagagtacagccactgcgcctggaccatcgtgagggtggagatcctgcggaacttctacttcatcaacaggctgaccggctacctgaggaactgatgagtccgcggccgc

SEQ ID NO: 28 - DNA, 763 bp, Artificial Sequence
  CTP-modified IFN
tctagaggacatgaccaacaagtgcctgctgcagatcgccctgctgctgtgcttcagcaccaccgccctgagcagcagcagctccaaggccccaccccccagcctgcccagccccagcagactgccaggccccagcgacacccccatcctgccccagatgagctacaacctgctgggcttcctgcagaggtccagcaacttccagtgccagaagctgctgtggcagctgaacggcaggctggaatactgcctgaaggacaggatgaacttcgacatcccagaggaaatcaagcagctgcagcagttccagaaggaggacgccgccctgaccatctacgagatgctgcagaacatcttcgccatcttcaggcaggacagcagcagcaccggctggaacgagaccatcgtggagaacctgctggccaacgtgtaccaccagatcaaccacctgaaaaccgtgctggaagagaagctggaaaaggaggacttcaccaggggcaagctgatgagcagcctgcacctgaagaggtactacggcagaatcctgcactacctgaaggccaaggagtacagccactgcgcctggaccatcgtgagggtggagatcctgaggaacttctacttcatcaacaggctgaccggctacctgaggaacagctccagcagcaaggcccctccaccttccctgcccagtccaagccgactccctgggccctccgatacaccaattctgccacagtgatgaaggtctggatgcggccgc

SEQ ID NO: 29 - protein, 166 aa, Artificial Sequence; identical to SEQ ID NO: 20
  IFN-beta

SEQ ID NO: 30 - DNA, 1356 bp, Artificial Sequence
  FVII
ctcgaggacatggtctcccaggccctcaggctcctctgccttctgcttgggcttcagggctgcctggctgcagtcttcgtaacccaggaggaagcccacggcgtcctgcaccggcgccggcgcgccaacgcgttcctggaggagctgcggccgggctccctggagagggagtgcaaggaggagcagtgctccttcgaggaggcccgggagatcttcaaggacgcggagaggacgaagctgttctggatttcttacagtgatggggaccagtgtgcctcaagtccatgccagaatgggggctcctgcaaggaccagctccagtcctatatctgcttctgcctccctgccttcgagggccggaactgtgagacgcacaaggatgaccagctgatctgtgtgaacgagaacggcggctgtgagcagtactgcagtgaccacacgggcaccaagcgctcctgtcggtgccacgaggggtactctctgctggcagacggggtgtcctgcacacccacagttgaatatccatgtggaaaaatacctattctagaaaaaagaaatgccagcaaaccccaaggccgaattgtggggggcaaggtgtgccccaaaggggagtgtccatggcaggtcctgttgttggtgaatggagctcagttgtgtggggggaccctgatcaacaccatctgggtggtctccgcggcccactgtttcgacaaaatcaagaactggaggaacctgatcgcggtgctgggcgagcacgacctcagcgagcacgacggggatgagcagagccggcgggtggcgcaggtcatcatccccagcacgtacgtcccgggcaccaccaaccacgacatcgcgctgctccgcctgcaccagcccgtggtcctcactgaccatgtggtgcccctctgcctgcccgaacggacgttctctgagaggacgctggccttcgtgcgcttctcattggtcagcggctggggccagctgctggaccgtggcgccacggccctggagctcatggtcctcaacgtgccccggctgatgacccaggactgcctgcagcagtcacggaaggtgggagactccccaaatatcacggagtacatgttctgtgccggctactcggatggcagcaaggactcctgcaagggggacagtggaggcccacatgccacccactaccggggcacgtggtacctgacgggcatcgtcagctggggccagggctgcgcaaccgtgggccactttggggtgtacaccagggtctcccagtacatcgagtggctgcaaaagctcatgcgctcagagccacgcccaggagtcctcctgcgagccccatttccctgaggatgcggccgc

SEQ ID NO: 31 - protein, 444 aa, Artificial Sequence
  FVII
MVSQALRLLCLLLGLQGCLAAVFVTQEEAHGVLHRRRRANAFLEELRPGSLERECKEEQCSFEEAREIFKDAERTKLFWISYSDGDQCASSPCQNGGSCKDQLQSYICFCLPAFEGRNCETHKDDQLICVNENGGCEQYCSDHTGTKRSCRCHEGYSLLADGVSCTPTVEYPCGKIPILEKRNASKPQGRIVGGKVCPKGECPWQVLLLVNGAQLCGGTLINTIWVVSAAHCFDKIKNWRNLIAVLGEHDLSEHDGDEQSRRVAQVIIPSTYVPGTTNHDIALLRLHQPVVLTDHVVPLCLPERTFSERTLAFVRFSLVSGWGQLLDRGATALELMVLNVPRLMTQDCLQQSRKVGDSPNITEYMFCAGYSDGSKDSCKGDSGGPHATHYRGTWYLTGIVSWGQGCATVGHFGVYTRVSQYIEWLQKLMRSEPRPGVLLRAPFP

SEQ ID NO: 32 - protein, 448 aa, Artificial Sequence
  FVII
MVSQALRLLCLLLGLQGCLAAVFVTQEEAHGVLHRRRRANAFLEELRPGSLERECKEEQCSFEEAREIFKDAERTKLFWISYSDGDQCASSPCQNGGSCKDQLQSYICFCLPAFEGRNCETHKDDQLICVNENGGCEQYCSDHTGTKRSCRCHEGYSLLADGVSCTPTVEYPCGKIPILEKRNASKPQGRIVGGKVCPKGECPWQVLLLVNGAQLCGGTLINTIWVVSAAHCFDKIKNWRNLIAVLGEHDLSEHDGDEQSRRVAQVIIPSTYVPGTTNHDIALLRLHQPVVLTDHVVPLCLPERTFSERTLAFVRFSLVSGWGQLLDRGATALELMVLNVPRLMTQDCLQQSRKVGDSPNITEYMFCAGYSDGSKDSCKGDSGGPHATHYRGTWYLTGIVSWGQGCATVGHFGVYTRVSQYIEWLQKLMRSEPRPGVLLRAPFPGCGR

SEQ ID NO: 33 - DNA, 1442 bp, Artificial Sequence
  FVII-CTP
ctcgaggacatggtctcccaggccctcaggctcctctgccttctgcttgggcttcagggctgcctggctgcagtcttcgtaacccaggaggaagcccacggcgtcctgcaccggcgccggcgcgccaacgcgttcctggaggagctgcggccgggctccctggagagggagtgcaaggaggagcagtgctccttcgaggaggcccgggagatcttcaaggacgcggagaggacgaagctgttctggatttcttacagtgatggggaccagtgtgcctcaagtccatgccagaatgggggctcctgcaaggaccagctccagtcctatatctgcttctgcctccctgccttcgagggccggaactgtgagacgcacaaggatgaccagctgatctgtgtgaacgagaacggcggctgtgagcagtactgcagtgaccacacgggcaccaagcgctcctgtcggtgccacgaggggtactctctgctggcagacggggtgtcctgcacacccacagttgaatatccatgtggaaaaatacctattctagaaaaaagaaatgccagcaaaccccaaggccgaattgtggggggcaaggtgtgccccaaaggggagtgtccatggcaggtcctgttgttggtgaatggagctcagttgtgtggggggaccctgatcaacaccatctgggtggtctccgcggcccactgtttcgacaaaatcaagaactggaggaacctgatcgcggtgctgggcgagcacgacctcagcgagcacgacggggatgagcagagccggcgggtggcgcaggtcatcatccccagcacgtacgtcccgggcaccaccaaccacgacatcgcgctgctccgcctgcaccagcccgtggtcctcactgaccatgtggtgcccctctgcctgcccgaacggacgttctctgagaggacgctggccttcgtgcgcttctcattggtcagcggctggggccagctgctggaccgtggcgccacggccctggagctcatggtcctcaacgtgccccggctgatgacccaggactgcctgcagcagtcacggaaggtgggagactccccaaatatcacggagtacatgttctgtgccggctactcggatggcagcaaggactcctgcaagggggacagtggaggcccacatgccacccactaccggggcacgtggtacctgaccggcatcgtgagctggggccagggctgcgccaccgtgggccacttcggcgtgtacaccagggtgtcccagtacatcgagtggctgcagaaactgatgagaagcgagcccagacccggcgtgctgctgagagcccccttccccagcagcagctccaaggcccctccccctagcctgcccagccctagcagactgcctgggcccagcgacacccccatcctgccccagtgaggatccgcggccgc

SEQ ID NO: 34 - protein, 472 aa, Artificial Sequence
  FVII-CTP
MVSQALRLLCLLLGLQGCLAAVFVTQEEAHGVLHRRRRANAFLEELRPGSLERECKEEQCSFEEAREIFKDAERTKLFWISYSDGDQCASSPCQNGGSCKDQLQSYICFCLPAFEGRNCETHKDDQLICVNENGGCEQYCSDHTGTKRSCRCHEGYSLLADGVSCTPTVEYPCGKIPILEKRNASKPQGRIVGGKVCPKGECPWQVLLLVNGAQLCGGTLINTIWVVSAAHCFDKIKNWRNLIAVLGEHDLSEHDGDEQSRRVAQVIIPSTYVPGTTNHDIALLRLHQPVVLTDHVVPLCLPERTFSERTLAFVRFSLVSGWGQLLDRGATALELMVLNVPRLMTQDCLQQSRKVGDSPNITEYMFCAGYSDGSKDSCKGDSGGPHATHYRGTWYLTGIVSWGQGCATVGHFGVYTRVSQYIEWLQKLMRSEPRPGVLLRAPFPSSSSKAPPPSLPSPSRLPGPSDTPILPQ

SEQ ID NO: 35 - DNA, 1535 bp, Artificial Sequence
  FVII-CTP-CTP
ctcgaggacatggtctcccaggccctcaggctcctctgccttctgcttgggcttcagggctgcctggctgcagtcttcgtaacccaggaggaagcccacggcgtcctgcaccggcgccggcgcgccaacgcgttcctggaggagctgcggccgggctccctggagagggagtgcaaggaggagcagtgctccttcgaggaggcccgggagatcttcaaggacgcggagaggacgaagctgttctggatttcttacagtgatggggaccagtgtgcctcaagtccatgccagaatgggggctcctgcaaggaccagctccagtcctatatctgcttctgcctccctgccttcgagggccggaactgtgagacgcacaaggatgaccagctgatctgtgtgaacgagaacggcggctgtgagcagtactgcagtgaccacacgggcaccaagcgctcctgtcggtgccacgaggggtactctctgctggcagacggggtgtcctgcacacccacagttgaatatccatgtggaaaaatacctattctagaaaaaagaaatgccagcaaaccccaaggccgaattgtggggggcaaggtgtgccccaaaggggagtgtccatggcaggtcctgttgttggtgaatggagctcagttgtgtggggggaccctgatcaacaccatctgggtggtctccgcggcccactgtttcgacaaaatcaagaactggaggaacctgatcgcggtgctgggcgagcacgacctcagcgagcacgacggggatgagcagagccggcgggtggcgcaggtcatcatccccagcacgtacgtcccgggcaccaccaaccacgacatcgcgctgctccgcctgcaccagcccgtggtcctcactgaccatgtggtgcccctctgcctgcccgaacggacgttctctgagaggacgctggccttcgtgcgcttctcattggtcagcggctggggccagctgctggaccgtggcgccacggccctggagctcatggtcctcaacgtgccccggctgatgacccaggactgcctgcagcagtcacggaaggtgggagactccccaaatatcacggagtacatgttctgtgccggctactcggatggcagcaaggactcctgcaagggggacagtggaggcccacatgccacccactaccggggcacgtggtacctgaccggcatcgtgagctggggccagggctgcgccaccgtgggccacttcggcgtgtacaccagggtgtcccagtacatcgagtggctgcagaaactgatgagaagcgagcccagacccggcgtgctgctgagagcccccttccccagcagcagctccaaggcccctccccctagcctgcccagccctagcagactgcctgggccctccgacacaccaatcctgccacagagcagctcctctaaggcccctcctccatccctgccatccccctcccggctgccaggcccctctgacacccctatcctgcctcagtgatgaaggtctggatccgcggccgc

SEQ ID NO: 36 - protein, 500 aa, Artificial Sequence
  FVII-CTP-CTP
MVSQALRLLCLLLGLQGCLAAVFVTQEEAHGVLHRRRRANAFLEELRPGSLERECKEEQCSFEEAREIFKDAERTKLFWISYSDGDQCASSPCQNGGSCKDQLQSYICFCLPAFEGRNCETHKDDQLICVNENGGCEQYCSDHTGTKRSCRCHEGYSLLADGVSCTPTVEYPCGKIPILEKRNASKPQGRIVGGKVCPKGECPWQVLLLVNGAQLCGGTLINTIWVVSAAHCFDKIKNWRNLIAVLGEHDLSEHDGDEQSRRVAQVIIPSTYVPGTTNHDIALLRLHQPVVLTDHVVPLCLPERTFSERTLAFVRFSLVSGWGQLLDRGATALELMVLNVPRLMTQDCLQQSRKVGDSPNITEYMFCAGYSDGSKDSCKGDSGGPHATHYRGTWYLTGIVSWGQGCATVGHFGVYTRVSQYIEWLQKLMRSEPRPGVLLRAPFPSSSSKAPPPSLPSPSRLPGPSDTPILPQSSSSKAPPPSLPSPSRLPGPSDTPILPQ

SEQ ID NO: 37 - DNA, 1621 bp, Artificial Sequence
  FVII-CTP-CTP-CTP (MOD-5014) with SP
ctcgaggacatggtctcccaggccctcaggctcctctgccttctgcttgggcttcagggctgcctggctgcagtcttcgtaacccaggaggaagcccacggcgtcctgcaccggcgccggcgcgccaacgcgttcctggaggagctgcggccgggctccctggagagggagtgcaaggaggagcagtgctccttcgaggaggcccgggagatcttcaaggacgcggagaggacgaagctgttctggatttcttacagtgatggggaccagtgtgcctcaagtccatgccagaatgggggctcctgcaaggaccagctccagtcctatatctgcttctgcctccctgccttcgagggccggaactgtgagacgcacaaggatgaccagctgatctgtgtgaacgagaacggcggctgtgagcagtactgcagtgaccacacgggcaccaagcgctcctgtcggtgccacgaggggtactctctgctggcagacggggtgtcctgcacacccacagttgaatatccatgtggaaaaatacctattctagaaaaaagaaatgccagcaaaccccaaggccgaattgtggggggcaaggtgtgccccaaaggggagtgtccatggcaggtcctgttgttggtgaatggagctcagttgtgtggggggaccctgatcaacaccatctgggtggtctccgcggcccactgtttcgacaaaatcaagaactggaggaacctgatcgcggtgctgggcgagcacgacctcagcgagcacgacggggatgagcagagccggcgggtggcgcaggtcatcatccccagcacgtacgtcccgggcaccaccaaccacgacatcgcgctgctccgcctgcaccagcccgtggtcctcactgaccatgtggtgcccctctgcctgcccgaacggacgttctctgagaggacgctggccttcgtgcgcttctcattggtcagcggctggggccagctgctggaccgtggcgccacggccctggagctcatggtcctcaacgtgccccggctgatgacccaggactgcctgcagcagtcacggaaggtgggagactccccaaatatcacggagtacatgttctgtgccggctactcggatggcagcaaggactcctgcaagggggacagtggaggcccacatgccacccactaccggggcacgtggtacctgaccggcatcgtgagctggggccagggctgcgccaccgtgggccacttcggcgtgtacaccagggtgtcccagtacatcgagtggctgcagaaactgatgagaagcgagcccagacccggcgtgctgctgagagcccccttccccagcagcagctccaaggcccctccccctagcctgcccagccctagcagactgcctgggcccagtgacacccctatcctgcctcagtccagctccagcaaggccccaccccctagcctgccttctccttctcggctgcctggccccagcgatactccaattctgccccagtcctccagcagtaaggctccccctccatctctgccatcccccagcagactgccaggcccttctgatacacccatcctcccacagtgatgaggatccgcggccgcttaattaa

SEQ ID NO: 38 - protein, 528 aa, Artificial Sequence
  FVII-CTP-CTP-CTP (MOD-5014) with Signal Peptide
MVSQALRLLCLLLGLQGCLAAVFVTQEEAHGVLHRRRRANAFLEELRPGSLERECKEEQCSFEEAREIFKDAERTKLFWISYSDGDQCASSPCQNGGSCKDQLQSYICFCLPAFEGRNCETHKDDQLICVNENGGCEQYCSDHTGTKRSCRCHEGYSLLADGVSCTPTVEYPCGKIPILEKRNASKPQGRIVGGKVCPKGECPWQVLLLVNGAQLCGGTLINTIWVVSAAHCFDKIKNWRNLIAVLGEHDLSEHDGDEQSRRVAQVIIPSTYVPGTTNHDIALLRLHQPVVLTDHVVPLCLPERTFSERTLAFVRFSLVSGWGQLLDRGATALELMVLNVPRLMTQDCLQQSRKVGDSPNITEYMFCAGYSDGSKDSCKGDSGGPHATHYRGTWYLTGIVSWGQGCATVGHFGVYTRVSQYIEWLQKLMRSEPRPGVLLRAPFPSSSSKAPPPSLPSPSRLPGPSDTPILPQSSSSKAPPPSLPSPSRLPGPSDTPILPQSSSSKAPPPSLPSPSRLPGPSDTPILPQ

SEQ ID NO: 39 - DNA, 1607 bp, Artificial Sequence
  FVII-CTP4X
ctcgaggacatggtctcccaggccctcaggctcctctgccttctgcttgggcttcagggctgcctggctgcagtcttcgtaacccaggaggaagcccacggcgtcctgcaccggcgccggcgcgccaacgcgttcctggaggagctgcggccgggctccctggagagggagtgcaaggaggagcagtgctccttcgaggaggcccgggagatcttcaaggacgcggagaggacgaagctgttctggatttcttacagtgatggggaccagtgtgcctcaagtccatgccagaatgggggctcctgcaaggaccagctccagtcctatatctgcttctgcctccctgccttcgagggccggaactgtgagacgcacaaggatgaccagctgatctgtgtgaacgagaacggcggctgtgagcagtactgcagtgaccacacgggcaccaagcgctcctgtcggtgccacgaggggtactctctgctggcagacggggtgtcctgcacacccacagttgaatatccatgtggaaaaatacctattctagaaaaaagaaatgccagcaaaccccaaggccgaattgtggggggcaaggtgtgccccaaaggggagtgtccatggcaggtcctgttgttggtgaatggagctcagttgtgtggggggaccctgatcaacaccatctgggtggtctccgcggcccactgtttcgacaaaatcaagaactggaggaacctgatcgcggtgctgggcgagcacgacctcagcgagcacgacggggatgagcagagccggcgggtggcgcaggtcatcatccccagcacgtacgtcccgggcaccaccaaccacgacatcgcgctgctccgcctgcaccagcccgtggtcctcactgaccatgtggtgcccctctgcctgcccgaacggacgttctctgagaggacgctggccttcgtgcgcttctcattggtcagcggctggggccagctgctggaccgtggcgccacggccctggagctcatggtcctcaacgtgccccggctgatgacccaggactgcctgcagcagtcacggaaggtgggagactccccaaatatcacggagtacatgttctgtgccggctactcggatggcagcaaggactcctgcaagggggacagtggaggcccacatgccacccactaccggggcacgtggtacctgaccggcatcgtgagctggggccagggctgcgccaccgtgggccacttcggcgtgtacaccagggtgtcccagtacatcgagtggctgcagaaactgatgagaagcgagcccagacccggcgtgctgctgagagcccccttccccagcagcagctccaaggcccctccccctagcctgcccagccctagcagactgcctgggcccagtgacacccctatcctgcctcagtccagctccagcaaggccccaccccctagcctgccttctccttctcggctgcctggccccagcgatactccaattctgccccagtcctccagcagtaaggctccccctccatctctgccatcccccagcagactgccaggcccttctgatacacccatcctcccacagtgatgaggatccgc

SEQ ID NO: 40 - protein, 532 aa, Artificial Sequence
  FVII-CTP4x
LEDMVSQALRLLCLLLGLQGCLAAVFVTQEEAHGVLHRRRRANAFLEELRPGSLERECKEEQCSFEEAREIFKDAERTKLFWISYSDGDQCASSPCQNGGSCKDQLQSYICFCLPAFEGRNCETHKDDQLICVNENGGCEQYCSDHTGTKRSCRCHEGYSLLADGVSCTPTVEYPCGKIPILEKRNASKPQGRIVGGKVCPKGECPWQVLLLVNGAQLCGGTLINTIWVVSAAHCFDKIKNWRNLIAVLGEHDLSEHDGDEQSRRVAQVIIPSTYVPGTTNHDIALLRLHQPVVLTDHVVPLCLPERTFSERTLAFVRFSLVSGWGQLLDRGATALELMVLNVPRLMTQDCLQQSRKVGDSPNITEYMFCAGYSDGSKDSCKGDSGGPHATHYRGTWYLTGIVSWGQGCATVGHFGVYTRVSQYIEWLQKLMRSEPRPGVLLRAPFPSSSSKAPPPSLPSPSRLPGPSDTPILPQSSSSKAPPPSLPSPSRLPGPSDTPILPQSSSSKAPPPSLPSPSRLPGPSDTPILPQG

SEQ ID NO: 41 - DNA, 1775 bp, Artificial Sequence
  FVII-CTP5x
ctcgaggacatggtctcccaggccctcaggctcctctgccttctgcttgggcttcagggctgcctggctgcagtcttcgtaacccaggaggaagcccacggcgtcctgcaccggcgccggcgcgccaacgcgttcctggaggagctgcggccgggctccctggagagggagtgcaaggaggagcagtgctccttcgaggaggcccgggagatcttcaaggacgcggagaggacgaagctgttctggatttcttacagtgatggggaccagtgtgcctcaagtccatgccagaatgggggctcctgcaaggaccagctccagtcctatatctgcttctgcctccctgccttcgagggccggaactgtgagacgcacaaggatgaccagctgatctgtgtgaacgagaacggcggctgtgagcagtactgcagtgaccacacgggcaccaagcgctcctgtcggtgccacgaggggtactctctgctggcagacggggtgtcctgcacacccacagttgaatatccatgtggaaaaatacctattctagaaaaaagaaatgccagcaaaccccaaggccgaattgtggggggcaaggtgtgccccaaaggggagtgtccatggcaggtcctgttgttggtgaatggagctcagttgtgtggggggaccctgatcaacaccatctgggtggtctccgcggcccactgtttcgacaaaatcaagaactggaggaacctgatcgcggtgctgggcgagcacgacctcagcgagcacgacggggatgagcagagccggcgggtggcgcaggtcatcatccccagcacgtacgtcccgggcaccaccaaccacgacatcgcgctgctccgcctgcaccagcccgtggtcctcactgaccatgtggtgcccctctgcctgcccgaacggacgttctctgagaggacgctggccttcgtgcgcttctcattggtcagcggctggggccagctgctggaccgtggcgccacggccctggagctcatggtcctcaacgtgccccggctgatgacccaggactgcctgcagcagtcacggaaggtgggagactccccaaatatcacggagtacatgttctgtgccggctactcggatggcagcaaggactcctgcaagggggacagtggaggcccacatgccacccactaccggggcacgtggtacctgaccggcatcgtgagctggggccagggctgcgccaccgtgggccacttcggcgtgtacaccagggtgtcccagtacatcgagtggctgcagaaactgatgagaagcgagcccagacccggcgtgctgctgagagcccccttccccagcagcagctccaaggcccctccccctagcctgcccagccctagcagactgcctgggccctctgacacccctatcctgcctcagtccagctcctctaaggctccaccaccttccctgcctagcccttcaagactgccaggccctagcgatacaccaattctgccccagtcctccagcagcaaggctcccccacctagcctgccttctccatcaaggctgcctggcccatccgataccccaattttgcctcagagcagctctagcaaggcacctccccccagtctgccctctccaagcagactccctggcccttcagacactccaatcctcccacagtcctctagctctaaagctccacctcccagcctgcccagccctagtagactccccggaccttctgatacccccatcttgccccagtgatgaggatccgc

SEQ ID NO: 42 - protein, 589 aa, Artificial Sequence
  FVII-CTP5x
LEDMVSQALRLLCLLLGLQGCLAAVFVTQEEAHGVLHRRRRANAFLEELRPGSLERECKEEQCSFEEAREIFKDAERTKLFWISYSDGDQCASSPCQNGGSCKDQLQSYICFCLPAFEGRNCETHKDDQLICVNENGGCEQYCSDHTGTKRSCRCHEGYSLLADGVSCTPTVEYPCGKIPILEKRNASKPQGRIVGGKVCPKGECPWQVLLLVNGAQLCGGTLINTIWVVSAAHCFDKIKNWRNLIAVLGEHDLSEHDGDEQSRRVAQVIIPSTYVPGTTNHDIALLRLHQPVVLTDHVVPLCLPERTFSERTLAFVRFSLVSGWGQLLDRGATALELMVLNVPRLMTQDCLQQSRKVGDSPNITEYMFCAGYSDGSKDSCKGDSGGPHATHYRGTWYLTGIVSWGQGCATVGHFGVYTRVSQYIEWLQKLMRSEPRPGVLLRAPFPSSSSKAPPPSLPSPSRLPGPSDTPILPQSSSSKAPPPSLPSPSRLPGPSDTPILPQSSSSKAPPPSLPSPSRLPGPSDTPILPQSSSSKAPPPSLPSPSRLPGPSDTPILPQSSSSKAPPPSLPSPSRLPGPSDTPILPQGS

SEQ ID NO: 43 - DNA, 1404 bp, Artificial Sequence
  FIX
gcgatcgccatgcagcgcgtgaacatgatcatggcagaatcaccaggcctcatcaccattgccttttaggatatctactcagtgctgaatgtacagtttttcttgatcatgaaaacgccaacaaaattctgaatcggccaaagaggtataattcaggtaaattggaagagtttgttcaagggaaccttgagagagaatgtatggaagaaaagtgtagttttgaagaagcacgagaagtttttgaaaacactgaaagaacaactgaattttggaagcagtatgttgatggagatcagtgtgagtccaatccatgtttaaatggcggcagttgcaaggatgacattaattcctatgaatgttggtgtccctttggatttgaaggaaagaactgtgaattagatgtaacatgtaacattaagaatggcagatgcgagcagttttgtaaaaatagtgctgataacaaggtggtttgctcctgtactgagggatatcgacttgcagaaaaccagaagtcctgtgaaccagcagtgccatttccatgtggaagagtttctgtttcacaaacttctaagctcacccgtgctgagactgtttttcctgatgtggactatgtaaattctactgaagctgaaaccattttggataacatcactcaaagcacccaatcatttaatgacttcactcgagttgttggtggagaagatgccaaaccaggtcaattcccttggcaggttgttttgaatggtaaagttgatgcattctgtggaggctctatcgttaatgaaaaatggattgtaactgctgcccactgtgttgaaactggtgttaaaattacagttgtcgcaggtgaacataatattgaggagacagaacatacagagcaaaagcgaaatgtgattcgaattattcctcaccacaactacaatgcagctattaataagtacaaccatgacattgcccttctggaactggacgaacccttagtgctaaacagctacgttacacctatttgcattgctgacaaggaatacacgaacatcttcctcaaatttggatctggctatgtaagtggctggggaagagtcttccacaaagggagatcagctttagttctccagtaccttagagttccacttgttgaccgagccacatgtcttcgatctacaaagttcaccatctataacaacatgttctgtgctggcttccatgaaggaggtagagattcatgtcaaggagatagtgggggaccccatgttactgaagtggaagggaccagtttcttaactggaattattagctggggtgaagagtgtgcaatgaaaggcaaatatggaatatataccaaggtatcccggtatgtcaactggattaaggaaaaaacaaagctcacttgaacgcggccgc

SEQ ID NO: 44 - protein, 461 aa, Artificial Sequence
  FIX
MQRVNMIMAESPGLITICLLGYLLSAECTVFLDHENANKILNRPKRYNSGKLEEFVQGNLERECMEEKCSFEEAREVFENTERTTEFWKQYVDGDQCESNPCLNGGSCKDDINSYECWCPFGFEGKNCELDVTCNIKNGRCEQFCKNSADNKVVCSCTEGYRLAENQKSCEPAVPFPCGRVSVSQTSKLTRAETVFPDVDYVNSTEAETILDNITQSTQSFNDFTRVVGGEDAKPGQFPWQVVLNGKVDAFCGGSIVNEKWIVTAAHCVETGVKITVVAGEHNIEETEHTEQKRNVIRIIPHHNYNAAINKYNHDIALLELDEPLVLNSYVTPICIADKEYTNIFLKFGSGYVSGWGRVFHKGRSALVLQYLRVPLVDRATCLRSTKFTIYNNMFCAGFHEGGRDSCQGDSGGPHVTEVEGTSFLTGIISWGEECAMKGKYGIYTKVSRYVNWIKEKTKLT

SEQ ID NO: 45 - DNA, 1502 bp, Artificial Sequence
  FIX-CTP
gcgatcgccatgcagcgcgtgaacatgatcatggcagaatcaccaggcctcatcaccatctgccttttaggatatctactcagtgctgaatgtacagtttttcttgatcatgaaaacgccaacaaaattctgaatcggccaaagaggtataattcaggtaaattggaagagtttgttcaagggaaccttgagagagaatgtatggaagaaaagtgtagttttgaagaagcacgagaagtttttgaaaacactgaaagaacaactgaattttggaagcagtatgttgatggagatcagtgtgagtccaatccatgtttaaatggcggcagttgcaaggatgacattaattcctatgaatgttggtgtccctttggatttgaaggaaagaactgtgaattagatgtaacatgtaacattaagaatggcagatgcgagcagttttgtaaaaatagtgctgataacaaggtggtttgctcctgtactgagggatatcgacttgcagaaaaccagaagtcctgtgaaccagcagtgccatttccatgtggaagagtttctgtttcacaaacttctaagctcacccgtgctgagactgtttttcctgatgtggactatgtaaattctactgaagctgaaaccattttggataacatcactcaaagcacccaatcatttaatgacttcactcgagttgttggtggagaagatgccaaaccaggtcaattcccttggcaggttgttttgaatggtaaagttgatgcattctgtggaggctctatcgttaatgaaaaatggattgtaactgctgcccactgtgttgaaactggtgttaaaattacagttgtcgcaggtgaacataatattgaggagacagaacatacagagcaaaagcgaaatgtgattcgaattattcctcaccacaactacaatgcagctattaataagtacaaccatgacattgcccttctggaactggacgaacccttagtgctaaacagctacgttacacctatttgcattgctgacaaggaatacacgaacatcttcctcaaatttggatctggctatgtaagtggctggggaagagtcttccacaaagggagatcagctttagttcttcagtaccttagagttccacttgttgaccgagccacatgtcttcgatctacaaagttcaccatctataacaacatgttctgtgctggcttccatgaaggaggtagagattcatgtcaaggagatagtgggggaccccatgttactgaagtggaagggaccagtttcttaactggaattattagctggggtgaagagtgtgcaatgaaaggcaaatatggaatatataccaaggtatcccggtatgtcaactggattaaggaaaaaacaaagctcactagctccagcagcaaggcccctcccccgagcctgccctccccaagcaggctgcctgggccctccgacacaccaatcctgccacagtgatgaaggtctggatccgcggccgc

SEQ ID NO: 46 - protein, 489 aa, Artificial Sequence
  FIX-CTP
MQRVNMIMAESPGLITICLLGYLLSAECTVFLDHENANKILNRPKRYNSGKLEEFVQGNLERECMEEKCSFEEAREVFENTERTTEFWKQYVDGDQCESNPCLNGGSCKDDINSYECWCPFGFEGKNCELDVTCNIKNGRCEQFCKNSADNKVVCSCTEGYRLAENQKSCEPAVPFPCGRVSVSQTSKLTRAETVFPDVDYVNSTEAETILDNITQSTQSFNDFTRVVGGEDAKPGQFPWQVVLNGKVDAFCGGSIVNEKWIVTAAHCVETGVKITVVAGEHNIEETEHTEQKRNVIRIIPHHNYNAAINKYNHDIALLELDEPLVLNSYVTPICIADKEYTNIFLKFGSGYVSGWGRVFHKGRSALVLQYLRVPLVDRATCLRSTKFTIYNNMFCAGFHEGGRDSCQGDSGGPHVTEVEGTSFLTGIISWGEECAMKGKYGIYTKVSRYVNWIKEKTKLTSSSSKAPPPSLPSPSRLPGPSDTPILPQ

SEQ ID NO: 47 - DNA, 1585 bp, Artificial Sequence
  FIX-CTP-CTP
gcgatcgccatgcagcgcgtgaacatgatcatggcagaatcaccaggcctcatcaccatctgccttttaggatatctactcagtgctgaatgtacagtttttcttgatcatgaaaacgccaacaaaattctgaatcggccaaagaggtataattcaggtaaattggaagagtttgttcaagggaaccttgagagagaatgtatggaagaaaagtgtagttttgaagaagcacgagaagtttttgaaaacactgaaagaacaactgaattttggaagcagtatgttgatggagatcagtgtgagtccaatccatgtttaaatggcggcagttgcaaggatgacattaattcctatgaatgttggtgtccctttggatttgaaggaaagaactgtgaattagatgtaacatgtaacattaagaatggcagatgcgagcagttttgtaaaaatagtgctgataacaaggtggtttgctcctgtactgagggatatcgacttgcagaaaaccagaagtcctgtgaaccagcagtgccatttccatgtggaagagtttctgtttcacaaacttctaagctcacccgtgctgagactgtttttcctgatgtggactatgtaaattctactgaagctgaaaccattttggataacatcactcaaagcacccaatcatttaatgacttcactcgagttgttggtggagaagatgccaaaccaggtcaattcccttggcaggttgttttgaatggtaaagttgatgcattctgtggaggctctatcgttaatgaaaaatggattgtaactgctgcccactgtgttgaaactggtgttaaaattacagttgtcgcaggtgaacataatattgaggagacagaacatacagagcaaaagcgaaatgtgattcgaattattcctcaccacaactacaatgcagctattaataagtacaaccatgacattgcccttctggaactggacgaacccttagtgctaaacagctacgttacacctatttgcattgctacaaggaatacacgaacatcttcctcaaatttggatctggctatgtaagtggctggggaagagtcttccacaaagggagatcagctttagttcttcagtaccttagagttccacttgttgaccgagccacatgtcttcgatctacaaagttcaccatctataacaacatgttctgtgctggcttccatgaaggaggtagagattcatgtcaaggagatagtgggggaccccatgttactgaagtggaagggaccagtttcttaactggaattattagctggggtgaagagtgtgcaatgaaaggcaaatatggaatatataccaaggtatcccggtatgtcaactggattaaggaaaaaacaaagctcactagctccagcagcaaggcccctcccccgagcctgccctccccaagcaggctgcctgggccctccgacacaccaatcctgccacagagcagctcctctaaggcccctcctccatccctgccatccccctcccggctgcctggcccctctgacacccctatcctgcctcagtgatgaaggtctggatccgcggccgc

SEQ ID NO: 48 - protein, 517 aa, Artificial Sequence
  FIX-CTP-CTP
MQRVNMIMAESPGLITICLLGYLLSAECTVFLDHENANKILNRPKRYNSGKLEEFVQGNLERECMEEKCSFEEAREVFENTERTTEFWKQYVDGDQCESNPCLNGGSCKDDINSYECWCPFGFEGKNCELDVTCNIKNGRCEQFCKNSADNKVVCSCTEGYRLAENQKSCEPAVPFPCGRVSVSQTSKLTRAETVFPDVDYVNSTEAETILDNITQSTQSFNDFTRVVGGEDAKPGQFPWQVVLNGKVDAFCGGSIVNEKWIVTAAHCVETGVKITVVAGEHNIEETEHTEQKRNVIRIIPHHNYNAAINKYNHDIALLELDEPLVLNSYVTPICIADKEYTNIFLKFGSGYVSGWGRVFHKGRSALVLQYLRVPLVDRATCLRSTKFTIYNNMFCAGFHEGGRDSCQGDSGGPHVTEVEGTSFLTGIISWGEECAMKGKYGIYTKVSRYVNWIKEKTKLTSSSSKAPPPSLPSPSRLPGPSDTPILPQSSSSKAPPPSLPSPSRLPGPSDTPILPQ

SEQ ID NO: 49 - DNA, 1673 bp, Artificial Sequence
  FIX-CTP-CTP-CTP (MOD-3013) with SP
tctagagtcgaccccgccatgcagcgcgtgaacatgatcatggcagaatcaccaggcctcatcaccatctgccttttaggatatctactcagtgctgaatgtacagtttttcttgatcatgaaaacgccaacaaaattctgaatcggccaaagaggtataattcaggtaaattggaagagtttgttcaagggaaccttgagagagaatgtatggaagaaaagtgtagttttgaagaagcacgagaagtttttgaaaacactgaaagaacaactgaattttggaagcagtatgttgatggagatcagtgtgagtccaatccatgtttaaatggcggcagttgcaaggatgacattaattcctatgaatgttggtgtccctttggatttgaaggaaagaactgtgaattagatgtaacatgtaacattaagaatggcagatgcgagcagttttgtaaaaatagtgctgataacaaggtggtttgctcctgtactgagggatatcgacttgcagaaaaccagaagtcctgtgaaccagcagtgccatttccatgtggaagagtttctgtttcacaaacttctaagctcacccgtgctgaggcagtttttcctgatgtggactatgtaaattctactgaagctgaaaccattttggataacatcactcaaagcacccaatcatttaatgacttcactcgagttgttggtggagaagatgccaaaccaggtcaattcccttggcaggttgttttgaatggtaaagttgatgcattctgtggaggctctatcgttaatgaaaaatggattgtaactgctgcccactgtgttgaaactggtgttaaaattacagttgtcgcaggtgaacataatattgaggagacagaacatacagagcaaaagcgaaatgtgattcgaattattcctcaccacaactacaatgcagctattaataagtacaaccatgacattgcccttctggaactggacgaacccttagtgctaaacagctacgttacacctatttgcattgctgacaaggaatacacgaacatcttcctcaaatttggatctggctatgtaagtggctggggaagagtcttccacaaagggagatcagctttagttcttcagtaccttagagttccacttgttgaccgagccacatgtcttcgatctacaaagttcaccatctataacaacatgttctgtgctggcttccatgaaggaggtagagattcatgtcaaggagatagtgggggaccccatgttactgaagtggaagggaccagtttcttaactggaattattagctggggtgaagagtgtgcaatgaaaggcaaatatggaatatataccaaggtatcccggtatgtcaactggattaaggaaaaaacaaagctcactagctccagcagcaaggcccctcccccgagcctgccctccccaagcaggctgcctgggcccagtgacacccctatcctgcctcagtccagctccagcaaggccccaccccctagcctgccttctccttctcggctgcctggccccagcgatactccaattctgccccagtcctccagcagtaaggctccccctccatctctgccatcccccagcagactgccaggcccttctgatacacccatcctcccacagtgatgaggatccgcggccgc

SEQ ID NO: 50 - protein, 545 aa, Artificial Sequence
  FIX-CTP-CTP-CTP (MOD-3013) with SP
MQRVNMIMAESPGLITICLLGYLLSAECTVFLDHENANKILNRPKRYNSGKLEEFVQGNLERECMEEKCSFEEAREVFENTERTTEFWKQYVDGDQCESNPCLNGGSCKDDINSYECWCPFGFEGKNCELDVTCNIKNGRCEQFCKNSADNKVVCSCTEGYRLAENQKSCEPAVPFPCGRVSVSQTSKLTRAEAVFPDVDYVNSTEAETILDNITQSTQSFNDFTRVVGGEDAKPGQFPWQVVLNGKVDAFCGGSIVNEKWIVTAAHCVETGVKITVVAGEHNIEETEHTEQKRNVIRIIPHHNYNAAINKYNHDIALLELDEPLVLNSYVTPICIADKEYTNIFLKFGSGYVSGWGRVFHKGRSALVLQYLRVPLVDRATCLRSTKFTIYNNMFCAGFHEGGRDSCQGDSGGPHVTEVEGTSFLTGIISWGEECAMKGKYGIYTKVSRYVNWIKEKTKLTSSSSKAPPPSLPSPSRLPGPSDTPILPQSSSSKAPPPSLPSPSRLPGPSDTPILPQSSSSKAPPPSLPSPSRLPGPSDTPILPQ

SEQ ID NO: 51 - DNA, 1757 bp, Artificial Sequence
  FIX-CTP4x
tctagagtcgaccccgccatgcagcgcgtgaacatgatcatggcagaatcaccaggcctcatcaccatctgccttttaggatatctactcagtgctgaatgtacagtttttcttgatcatgaaaacgccaacaaaattctgaatcggccaaagaggtataattcaggtaaattggaagagtttgttcaagggaaccttgagagagaatgtatggaagaaaagtgtagttttgaagaagcacgagaagtttttgaaaacactgaaagaacaactgaattttggaagcagtatgttgatggagatcagtgtgagtccaatccatgtttaaatggcggcagttgcaaggatgacattaattcctatgaatgttggtgtccctttggatttgaaggaaagaactgtgaattagatgtaacatgtaacattaagaatggcagatgcgagcagttttgtaaaaatagtgctgataacaaggtggtttgctcctgtactgagggatatcgacttgcagaaaaccagaagtcctgtgaaccagcagtgccatttccatgtggaagagtttctgtttcacaaacttctaagctcacccgtgctgaggcagtttttcctgatgtggactatgtaaattctactgaagctgaaaccattttggataacatcactcaaagcacccaatcatttaatgacttcactcgagttgttggtggagaagatgccaaaccaggtcaattcccttggcaggttgttttgaatggtaaagttgatgcattctgtggaggctctatcgttaatgaaaaatggattgtaactgctgcccactgtgttgaaactggtgttaaaattacagttgtcgcaggtgaacataatattgaggagacagaacatacagagcaaaagcgaaatgtgattcgaattattcctcaccacaactacaatgcagctattaataagtacaaccatgacattgcccttctggaactggacgaacccttagtgctaaacagctacgttacacctatttgcattgctgacaaggaatacacgaacatcttcctcaaatttggatctggctatgtaagtggctggggaagagtcttccacaaagggagatcagctttagttcttcagtaccttagagttccacttgttgaccgagccacatgtcttcgatctacaaagttcaccatctataacaacatgttctgtgctggcttccatgaaggaggtagagattcatgtcaaggagatagtgggggaccccatgttactgaagtggaagggaccagtttcttaactggaattattagctggggtgaagagtgtgcaatgaaaggcaaatatggaatatataccaaggtatcccggtatgtcaactggattaaggaaaaaacaaagctcactagctccagcagcaaggcccctcccccgagcctgccctccccaagcaggctgcctgggccctctgacacccctatcctgcctcagtccagctcctctaaggccccaccaccttccctgcctagcccttcaagactgccaggccctagcgatacaccaattctgccccagtcctccagcagcaaggctcccccacctagcctgccttctccatcaaggctgcctggcccatccgataccccaattttgcctcagagcagctctagcaaggcacctccccccagtctgccctctccaagcagactccctggcccttcagacactcccattctgccacagtgatgaggatccgcggccgc

SEQ ID NO: 52 - protein, 583 aa, Artificial Sequence
  FIX-CTP4x
SRVDPAMQRVNMIMAESPGLITICLLGYLLSAECTVFLDHENANKILNRPKRYNSGKLEEFVQGNLERECMEEKCSFEEAREVFENTERTTEFWKQYVDGDQCESNPCLNGGSCKDDINSYECWCPFGFEGKNCELDVTCNIKNGRCEQFCKNSADNKVVCSCTEGYRLAENQKSCEPAVPFPCGRVSVSQTSKLTRAEAVFPDVDYVNSTEAETILDNITQSTQSFNDFTRVVGGEDAKPGQFPWQVVLNGKVDAFCGGSIVNEKWIVTAAHCVETGVKITVVAGEHNIEETEHTEQKRNVIRIIPHHNYNAAINKYNHDIALLELDEPLVLNSYVTPICIADKEYTNIFLKFGSGYVSGWGRVFHKGRSALVLQYLRVPLVDRATCLRSTKFTIYNNMFCAGFHEGGRDSCQGDSGGPHVTEVEGTSFLTGIISWGEECAMKGKYGIYTKVSRYVNWIKEKTKLTSSSSKAPPPSLPSPSRLPGPSDTPILPQSSSSKAPPPSLPSPSRLPGPSDTPILPQSSSSKAPPPSLPSPSRLPGPSDTPILPQSSSSKAPPPSLPSPSRLPGPSDTPILPQGSAA

SEQ ID NO: 53 - DNA, 1840 bp, Artificial Sequence
  FIX-CTP5x
ctagagtcgaccccgccatgcagcgcgtgaacatgatcatggcagaatcaccaggcctcatcaccatctgccttttaggatatctactcagtgctgaatgtacagtttttcttgatcatgaaaacgccaacaaaattctgaatcggccaaagaggtataattcaggtaaattggaagagtttgttcaagggaaccttgagagagaatgtatggaagaaaagtgtagttttgaagaagcacgagaagtttttgaaaacactgaaagaacaactgaattttggaagcagtatgttgatggagatcagtgtgagtccaatccatgtttaaatggcggcagttgcaaggatgacattaattcctatgaatgttggtgtccctttggatttgaaggaaagaactgtgaattagatgtaacatgtaacattaagaatggcagatgcgagcagttttgtaaaaatagtgctgataacaaggtggtttgctcctgtactgagggatatcgacttgcagaaaaccagaagtcctgtgaaccagcagtgccatttccatgtggaagagtttctgtttcacaaacttctaagctcacccgtgctgaggcagtttttcctgatgtggactatgtaaattctactgaagctgaaaccattttggataacatcactcaaagcacccaatcatttaatgacttcactcgagttgttggtggagaagatgccaaaccaggtcaattcccttggcaggttgttttgaatggtaaagttgatgcattctgtggaggctctatcgttaatgaaaaatggattgtaactgctgcccactgtgttgaaactggtgttaaaattacagttgtcgcaggtgaacataatattgaggagacagaacatacagagcaaaagcgaaatgtgattcgaattattcctcaccacaactacaatgcagctattaataagtacaaccatgacattgcccttctggaactggacgaacccttagtgctaaacagctacgttacacctatttgcattgctgacaaggaatacacgaacatcttcctcaaatttggatctggctatgtaagtggctggggaagagtcttccacaaagggagatcagctttagttcttcagtaccttagagttccacttgttgaccgagccacatgtcttcgatctacaaagttcaccatctataacaacatgttctgtgctggcttccatgaaggaggtagagattcatgtcaaggagatagtgggggaccccatgttactgaagtggaagggaccagtttcttaactggaattattagctggggtgaagagtgtgcaatgaaaggcaaatatggaatatataccaaggtatcccggtatgtcaactggattaaggaaaaaacaaagctcactagctccagcagcaaggcccctcccccgagcctgccctccccaagcaggctgcctgggccctctgacacccctatcctgcctcagtccagctcctctaaggctccaccaccttccctgcctagcccttcaagactgccaggccctagcgatacaccaattctgccccagtcctccagcagcaaggctcccccacctagcctgccttctccatcaaggctgcctggcccatccgataccccaattttgcctcagagcagctctagcaaggcacctccccccagtctgccctctccaagcagactccctggcccttcagacactccaatcctcccacagtcctctagctctaaagctccacctcccagcctgcccagccctagtagactccccggaccttctgatacccccatcttgccccagtgatgaggatccgcggccgc

SEQ ID NO: 54 - protein, 610 aa, Artificial Sequence [sequence omitted]

SEQ ID NO: 55 - DNA, 2413 bp, Artificial Sequence
  furin
tctagagtcgaccccgccatggagctgaggccctggttgctatgggtggtagcagcaacaggaaccttggtcctgctagcagctgatgctcagggccagaaggtcttcaccaacacgtgggctgtgcgcatccctggaggcccagcggtggccaacagtgtggcacggaagcatgggttcctcaacctgggccagatcttcggggactattaccacttctggcatcgaggagtgacgaagcggtccctgtcgcctcaccgcccgcggcacagccggctgcagagggagcctcaagtacagtggctggaacagcaggtggcaaagcgacggactaaacgggacgtgtaccaggagcccacagaccccaagtttcctcagcagtggtacctgtctggtgtcactcagcgggacctgaatgtgaaggcggcctgggcgcagggctacacagggcacggcattgtggtctccattctggacgatggcatcgagaagaaccacccggacttggcaggcaattatgatcctggggccagttttgatgtcaatgaccaggaccctgacccccagcctcggtacacacagatgaatgacaacaggcacggcacacggtgtgcgggggaagtggctgcggtggccaacaacggtgtctgtggtgtaggtgtggcctacaacgcccgcattggaggggtgcgcatgctggatggcgaggtgacagatgcagtggaggcacgctcgctgggcctgaaccccaaccacatccacatctacagtgccagctggggccccgaggatgacggcaagacagtggatgggccagcccgcctcgccgaggaggccttcttccgtggggttagccagggccgaggggggctgggctccatctttgtctgggcctcggggaacgggggccgggaacatgacagctgcaactgcgacggctacaccaacagtatctacacgctgtccatcagcagcgccacgcagtttggcaacgtgccgtggtacagcgaggcctgctcgtccacactggccacgacctacagcagtggcaaccagaatgagaagcagatcgtgacgactgacttgcggcagaagtgcacggagtctcacacgggcacctcagcctctgcccccttagcagccggcatcattgctctcaccctggaggccaataagaacctcacatggcgggacatgcaacacctggtggtacagacctcgaagccagcccacctcaatgccaacgactgggccaccaatggtgtgggccggaaagtgagccactcatatggctacgggcttttggacgcaggcgccatggtggccctggcccagaattggaccacagtggccccccagcggaagtgcatcatcgacatcctcaccgagcccaaagacatcgggaaacggctcgaggtgcggaagaccgtgaccgcgtgcctgggcgagcccaaccacatcactcggctggagcacgctcaggcgcggctcaccctgtcctataatcgccgtggcgacctggccatccacctggtcagccccatgggcacccgctccaccctgctggcagccaggccacatgactactccgcagatgggtttaatgactgggccttcatgacaactcattcctgggatgaggatccctctggcgagtgggtcctagagattgaaaacaccagcgaagccaacaactatgggacgctgaccaagttcaccctcgtactctatggcaccgcccctgaggggctgcccgtacctccagaaagcagtggctgcaagaccctcacgtccagtcaggcctgtgtggtgtgcgaggaaggcttctccctgcaccagaagagctgtgtccagcactgccctccaggcttcgccccccaagtcctcgatacgcactatagcaccgagaatgacgtggagaccatccgggccagcgtctgcgccccctgccacgcctcatgtgccacatgccaggggccggccctgacagactgcctcagctgccccagccacgcctccttggaccctgtggagcagacttgctcccggcaaagccagagcagccgagagtccccgccacagcagcagccacctcggctgcccccggaggtggaggcggggcaacggctgcgggcagggctgctgccctcacacctgcctgaggtggtggccggcctcagctgcgccttcatcgtgctggtcttcgtcactgtcttcctggtcctgcagctgcgctctggctttagttttcggggggtgaaggtgtacaccatggaccgtggcctcatctcctacaaggggctgccccctgaagcctggcaggaggagtgcccgtctgactcagaagaggacgagggccggggcgagaggaccgcctttatcaaagaccagagcgccctctgaacgcggccgc

SEQ ID NO: 56 - protein, 794 aa, Artificial Sequence
  furin
MELRPWLLWVVAATGTLVLLAADAQGQKVFTNTWAVRIPGGPAVANSVARKHGFLNLGQIFGDYYHFWHRGVTKRSLSPHRPRHSRLQREPQVQWLEQQVAKRRTKRDVYQEPTDPKFPQQWYLSGVTQRDLNVKAAWAQGYTGHGIVVSILDDGIEKNHPDLAGNYDPGASFDVNDQDPDPQPRYTQMNDNRHGTRCAGEVAAVANNGVCGVGVAYNARIGGVRMLDGEVTDAVEARSLGLNPNHIHIYSASWGPEDDGKTVDGPARLAEEAFFRGVSQGRGGLGSIFVWASGNGGREHDSCNCDGYTNSIYTLSISSATQFGNVPWYSEACSSTLATTYSSGNQNEKQIVTTDLRQKCTESHTGTSASAPLAAGIIALTLEANKNLTWRDMQHLVVQTSKPAHLNANDWATNGVGRKVSHSYGYGLLDAGAMVALAQNWTTVAPQRKCIIDILTEPKDIGKRLEVRKTVTACLGEPNHITRLEHAQARLTLSYNRRGDLAIHLVSPMGTRSTLLAARPHDYSADGFNDWAFMTTHSWDEDPSGEWVLEIENTSEANNYGTLTKFTLVLYGTAPEGLPVPPESSGCKTLTSSQACVVCEEGFSLHQKSCVQHCPPGFAPQVLDTHYSTENDVETIRASVCAPCHASCATCQGPALTDCLSCPSHASLDPVEQTCSRQSQSSRESPPQQQPPRLPPEVEAGQRLRAGLLPSHLPEVVAGLSCAFIVLVFVTVFLVLQLRSGFSFRGVKVYTMDRGLISYKGLPPEAWQEECPSDSEEDEGRGERTAFIKDQSAL

SEQ ID NO: 57 - protein, 37 aa, Artificial Sequence
  oxyntomodulin
HSQGTFTSDYSKYLDSRRAQDFVQWLMNTKRNRNNIA

SEQ ID NO: 58 - protein, 119 aa, Artificial Sequence
  CTP-OXM-CTP
MATGSRTSLLLAFGLLCLPWLQEGSASSSSKAPPPSLPSPSRLPGPSDTPILPQHSQGTFTSDYSKYLDSRRAQDFVQWLMNTKRNRNNIASSSSKAPPPSLPSPSRLPGPSDTPILPQ

SEQ ID NO: 59 - protein, 147 aa, Artificial Sequence
  CTP-OXM-CTP-CTP
MATGSRTSLLLAFGLLCLPWLQEGSASSSSKAPPPSLPSPSRLPGPSDTPILPQHSQGTFTSDYSKYLDSRRAQDFVQWLMNTKRNRNNIASSSSKAPPPSLPSPSRLPGPSDTPILPQSSSSKAPPPSLPSPSRLPGPSDTPILPQ

SEQ ID NO: 60 - protein, 122 aa, Artificial Sequence
  OXM-CTP-CTP
LEDMATGSRTSLLLAFGLLCLPWLQEGSAHSQGTFTSDYSKYLDSRRAQDFVQWLMNTKRNRNNIASSSSKAPPPSLPSPSRLPGPSDTPILPQSSSSKAPPPSLPSPSRLPGPSDTPILPQ

SEQ ID NO: 61 - protein, 140 aa, Artificial Sequence [sequence omitted]

SEQ ID NO: 62 - protein, 147 aa, Artificial Sequence
  OXM-CTP-CTP-CTP
MATGSRTSLLLAFGLLCLPWLQEGSAHSQGTFTSDYSKYLDSRRAQDFVQWLMNTKRNRNNIASSSSKAPPPSLPSPSRLPGPSDTPILPQSSSSKAPPPSLPSPSRLPGPSDTPILPQSSSSKAPPPSLPSPSRLPGPSDTPILPQ

SEQ ID NO: 63 - protein, 175 aa, Artificial Sequence
  OXM-CTP-4x
MATGSRTSLLLAFGLLCLPWLQEGSAHSQGTFTSDYSKYLDSRRAQDFVQWLMNTKRNRNNIASSSSKAPPPSLPSPSRLPGPSDTPILPQSSSSKAPPPSLPSPSRLPGPSDTPILPQSSSSKAPPPSLPSPSRLPGPSDTPILPQSSSSKAPPPSLPSPSRLPGPSDTPILPQ

SEQ ID NO: 64 - protein, 203 aa, Artificial Sequence
  OXM-CTP-5x
MATGSRTSLLLAFGLLCLPWLQEGSAHSQGTFTSDYSKYLDSRRAQDFVQWLMNTKRNRNNIASSSSKAPPPSLPSPSRLPGPSDTPILPQSSSSKAPPPSLPSPSRLPGPSDTPILPQSSSSKAPPPSLPSPSRLPGPSDTPILPQSSSSKAPPPSLPSPSRLPGPSDTPILPQSSSSKAPPPSLPSPSRLPGPSDTPILPQ

SEQ ID NO: 65 - DNA, 391 bp, Artificial Sequence
  CTP-OXM-CTP
tctagaggacatggccaccggcagcaggaccagcctgctgctggccttcggcctgctgtgcctgccatggctgcaggagggcagcgccagctcttcttctaaggctccacccccatctctgcccagccccagcagactgccgggccccagcgacacacccattctgccccagcacagccagggcaccttcaccagcgactacagcaagtacctggacagcagaagggcccaggacttcgtccagtggctgatgaacaccaagaggaacaggaacaacatcgcttcctctagctccaaggcccctccaccctctctgcctagcccctctcggctgcctggcccatccgacacaccaatcctgccacagtgatgaaggtctggatgcggccgc

SEQ ID NO: 66 - DNA, 475 bp, Artificial Sequence
  CTP-OXM-CTP-CTP
tctagaggacatggccaccggcagcaggaccagcctgctgctggccttcggcctgctgtgcctgccatggctgcaggagggcagcgccagctcttcttctaaggctccacccccatctctgcccagccccagcagactgccgggccccagcgacacacccattctgccccagcacagccagggcaccttcaccagcgactacagcaagtacctggacagcagaagggcccaggacttcgtccagtggctgatgaacaccaagaggaacaggaacaacatcgctagctccagcagcaaggcccctcccccgagcctgccctccccaagcaggctgcctgggccctccgacacaccaatcctgccacagagcagctcctctaaggcccctcctccatccctgccatccccctcccggctgcctggcccctctgacacccctatcctgcctcagtgatgaaggtctggatgcggccgc

SEQ ID NO: 67 - DNA, 391 bp, Artificial Sequence
  OXM-CTP-CTP
tctagaggacatggccacagggagcaggaccagcctgctgctggctttcggcctgctgtgtctgccatggctgcaggagggcagcgctcacagccagggcaccttcaccagcgactacagcaagtacctggacagcagaagggcccaggacttcgtccagtggctgatgaacaccaagaggaacaggaacaacatcgctagctccagcagcaaggcccctcccccgagcctgccctccccaagcaggctgcctgggccctccgacacaccaatcctgccacagagcagctcctctaaggcccctcctccatccctgccatccccctcccggctgcctggcccctctgacacccctatcctgcctcagtgatgaaggtctggatgcggccgc

SEQ ID NO: 68 - DNA, 481 bp, Artificial Sequence
  CTP-CTP-OXM
ctatagggcgaattgaaggaaggccgtcaaggccgcatgagctctctagaggacatggccaccggcagcaggaccagcctgctgctggccttcggcctgctgtgcctgccatggctgcaggagggcagcgccagctccagcagcaaggcccctcccccgagcctgccctccccaagcaggctgcctgggccctccgacacaccaatcctgccacagagcagctcctctaaggcccctcctccatccctgccatccccctcccggctgcctggcccctctgacacccctatcctgcctcagcacagccagggcaccttcaccagcgactacagcaagtacctggacagcagaagggcccaggacttcgtccagtggctgatgaacaccaagaggaacaggaacaacatcgcttgatgaaggtctggatgcggccgcggtaccctgggcctcatgggccttcctttcactgcccgctttccag

SEQ ID NO: 69 - DNA, 481 bp, Artificial Sequence
  OXM-CTP-CTP-CTP
tctagactcgagcgatcgccatggccaccggctctaggacctccctgctgctggccttcggcctgctgtgcctgccctggctgcaggaaggcagcgctcactcccagggcaccttcacctccgactactccaagtacctggactctcggagagcccaggacttcgtgcagtggctgatgaacaccaagcggaaccggaacaatatcgcctcctcaagctccaaggcacctccaccttccctgcctagcccttccagactccctgggcccagtgacacccctatcctgcctcagtccagctccagcaaggccccaccccctagcctgccttctccttctcggctgcctggccccagcgatactccaattctgccccagtcctccagcagtaaggctccccctccatctctgccatcccccagcagactgccaggcccttctgatacacccatcctcccacagtgatgaggatccgcggccgc

SEQ ID NO: 70 - DNA, 565 bp, Artificial Sequence
  OXM-CTP-4x
tctagactcgagcgatcgccatggctaccggctccagaacctctctgctgctggccttcggcctgctgtgtctgccttggctgcaagagggcagcgctcattcccagggcaccttcacctccgactactccaagtacctggactctcgcagagcccaggacttcgtgcagtggctgatgaacaccaagcggaaccggaacaatatcgcctcctccagctccaaggcccctcctccatctctgccatcccccagtagactgcctgggccctctgacacccctatcctgcctcagtccagctcctctaaggccccaccaccttccctgcctagcccttcaagactgccaggccctagcgatacaccaattctgccccagtcctccagcagcaaggctcccccacctagcctgccttctccatcaaggctgcctggcccatccgataccccaattttgcctcagagcagctctagcaaggcacctccccccagtctgccctctccaagcagactccctggcccttcagacactcccattctgccacagtgatgaggatccgcggccgc

SEQ ID NO: 71 - DNA, 650 bp, Artificial Sequence
  OXM-CTP-5x
ctctagactcgagcgatcgccatggctaccggctccagaacctctctgctgctggccttcggcctgctgtgtctgccttggctgcaagagggcagcgctcattcccagggcaccttcacctccgactactccaagtacctggactctcgcagagcacaggacttcgtgcagtggctgatgaacaccaagcggaaccggaacaatatcgcctcctccagctccaaggcccctcctccatctctgccatcccccagtagactgcctgggccctctgacacccctatcctgcctcagtccagctcctctaaggctccaccaccttccctgcctagcccttcaagactgccaggccctagcgatacaccaattctgccccagtcctccagcagcaaggctcccccacctagcctgccttctccatcaaggctgcctggcccatccgataccccaattttgcctcagagcagctctagcaaggcacctccccccagtctgccctctccaagcagactccctggcccttcagacactccaatcctcccacagtcctctagctctaaagctccacctcccagcctgcccagccctagtagactccccggaccttctgatacccccatcttgccccagtgatgaggatccgcggccgc

SEQ ID NO: 72 - DNA, 25 bp, Artificial Sequence
  Primer
aatctagaggtcatcatgggggtgc

SEQ ID NO: 73 - DNA, 32 bp, Artificial Sequence
  Primer
attgcggccgcggatccagaagacctttattg

SEQ ID NO: 74 - DNA, 25 bp, Artificial Sequence
  Primer
taaatattggggtgtccgagggccc

SEQ ID NO: 75 - DNA, 32 bp, Artificial Sequence
  Primer
ccaatattaccacaagccccaccacgcctcat

SEQ ID NO: 76 - DNA, 35 bp, Artificial Sequence
  Primer
tgcggccgcggatccttatctgtcccctgtcctgc

SEQ ID NO: 77 - DNA, 17 bp, Artificial Sequence
  Primer
gccctgctgtcggaagc

SEQ ID NO: 78 - DNA, 32 bp, Artificial Sequence; identical to SEQ ID NO: 73
  Primer

SEQ ID NO: 79 - DNA, 32 bp, Artificial Sequence
  Primer
ctttgaggaagaggagcccaggactgggaggc

SEQ ID NO: 80 - DNA, 24 bp, Artificial Sequence
  Primer
cctgggctcctcttcctcaaaggc

SEQ ID NO: 81 - DNA, 17 bp, Artificial Sequence
  Primer
gcttccgacagcagggc

SEQ ID NO: 82 - DNA, 20 bp, Artificial Sequence
  Primer
gtttagtgaaccgtcagaat

SEQ ID NO: 83 - DNA, 20 bp, Artificial Sequence
  Primer
ttgaggaagatgttcgtgta

SEQ ID NO: 84 - DNA, 20 bp, Artificial Sequence
  Primer
attacagttgtcgcaggtga

SEQ ID NO: 85 - DNA, 30 bp, Artificial Sequence
  Primer
gctggagctagtgagctttgttttttcctt

SEQ ID NO: 86 - DNA, 23 bp, Artificial Sequence
  Primer
ttttcactgcattctagttgtgg

SEQ ID NO: 87 - DNA, 20 bp, Artificial Sequence
  Primer
ctcccagttcaattacagct

SEQ ID NO: 88 - DNA, 27 bp, Artificial Sequence
  Primer
ggaaaaactgcctcagcacgggtgagc

SEQ ID NO: 89 - DNA, 32 bp, Artificial Sequence
  Primer
gtgctgaggcagtttttcctgatgtggactat

SEQ ID NO: 90 - DNA, 18 bp, Artificial Sequence
  Primer
caacacagtgggcagcag

SEQ ID NO: 91 - DNA, 25 bp, Artificial Sequence
  Primer
ctcgaggacatggtctcccaggccc

SEQ ID NO: 92 - DNA, 25 bp, Artificial Sequence
  Primer
tctagaataggtatttttccacatg

SEQ ID NO: 93 - DNA, 22 bp, Artificial Sequence
  Primer
tctagaaaaaagaaatgccagc

SEQ ID NO: 94 - DNA, 32 bp, Artificial Sequence
  Primer
gcggccgcatcctcagggaaatggggctcgca

SEQ ID NO: 95 - DNA, 19 bp, Artificial Sequence
  Primer
ctctagaggacatggccac

SEQ ID NO: 96 - DNA, 27 bp, Artificial Sequence
  Primer
ctggctgtgctggggcagaatgggtgt

SEQ ID NO: 97 - DNA, 17 bp, Artificial Sequence
  Primer
ccccagcacagccaggg

SEQ ID NO: 98 - DNA, 18 bp, Artificial Sequence
  Primer
gcggccgcatccagacct

SEQ ID NO: 99 - DNA, 19 bp, Artificial Sequence
  Primer
ctctagaggacatggccac

SEQ ID NO: 100 - DNA, 29 bp, Artificial Sequence
  Primer
gctggagctagcgatgttgttcctgttcc

SEQ ID NO: 101 - DNA, 26 bp, Artificial Sequence
  Primer
acatcgctagctccagcagcaaggcc

SEQ ID NO: 102 - DNA, 18 bp, Artificial Sequence
  Primer
gcggccgcatccagacct

SEQ ID NO: 103 - DNA, 20 bp, Artificial Sequence
  Primer
ctcccagttcaattacagct

SEQ ID NO: 104 - DNA, 24 bp, Artificial Sequence
  Primer
gctgtgagcgctgccctcctgcag

SEQ ID NO: 105 - DNA, 23 bp, Artificial Sequence
  Primer
gcgctcacagccagggcaccttc

SEQ ID NO: 106 - DNA, 18 bp, Artificial Sequence
  Primer
gcggccgcatccagacct

SEQ ID NO: 107 - DNA, 25 bp, Artificial Sequence
  Primer
gctcactagctccagcagcaaggcc

SEQ ID NO: 108 - protein, 21 aa, Artificial Sequence
  signal peptide IFN Beta1
MTNKCLLQIALLLCFSTTALS

SEQ ID NO: 109 - protein, 250 aa, Artificial Sequence
  CTP-modified EPO without the SP
SSSSKAPPPSLPSPSRLPGPSDTPILPQAPPRLICDSRVLERYLLEAKEAENITTGCAEHCSLNENITVPDTKVNFYAWKRMEVGQQAVEVWQGLALLSEAVLRGQALLVNSSQPWEPLQLHVDKAVSGLRSLTTLLRALGAQKEAISPPDAASAAPLRTITADTFRKLFRVYSNFLRGKLKLYTGEACRTGDRSSSSKAPPPSLPSPSRLPGPSDTPILPQSSSSKAPPPSLPSPSRLPGPSDTPILPQ

SEQ ID NO: 110 - protein, 38 aa, Artificial Sequence
  Signal peptide of FVII
MVSQALRLLCLLLGLQGCLAAVFVTQEEAHGVLHRRRR

SEQ ID NO: 111 - protein, 490 aa, Artificial Sequence
  CTP-modified FVII/FVIIa without SP MOD-5014
ANAFLEELRPGSLERECKEEQCSFEEAREIFKDAERTKLFWISYSDGDQCASSPCQNGGSCKDQLQSYICFCLPAFEGRNCETHKDDQLICVNENGGCEQYCSDHTGTKRSCRCHEGYSLLADGVSCTPTVEYPCGKIPILEKRNASKPQGRIVGGKVCPKGECPWQVLLLVNGAQLCGGTLINTIWVVSAAHCFDKIKNWRNLIAVLGEHDLSEHDGDEQSRRVAQVIIPSTYVPGTTNHDIALLRLHQPVVLTDHVVPLCLPERTFSERTLAFVRFSLVSGWGQLLDRGATALELMVLNVPRLMTQDCLQQSRKVGDSPNITEYMFCAGYSDGSKDSCKGDSGGPHATHYRGTWYLTGIVSWGQGCATVGHFGVYTRVSQYIEWLQKLMRSEPRPGVLLRAPFPSSSSKAPPPSLPSPSRLPGPSDTPILPQSSSSKAPPPSLPSPSRLPGPSDTPILPQSSSSKAPPPSLPSPSRLPGPSDTPILPQ

SEQ ID NO: 112 - protein, 46 aa, Artificial Sequence
  Signal peptide of FIX
MQRVNMIMAESPGLITICLLGYLLSAECTVFLDHENANKILNRPKR

SEQ ID NO: 113 - protein, 499 aa, Artificial Sequence
  CTP-modified FIX without SP MOD-3013
YNSGKLEEFVQGNLERECMEEKCSFEEAREVFENTERTTEFWKQYVDGDQCESNPCLNGGSCKDDINSYECWCPFGFEGKNCELDVTCNIKNGRCEQFCKNSADNKVVCSCTEGYRLAENQKSCEPAVPFPCGRVSVSQTSKLTRAEAVFPDVDYVNSTEAETILDNITQSTQSFNDFTRVVGGEDAKPGQFPWQVVLNGKVDAFCGGSIVNEKWIVTAAHCVETGVKITVVAGEHNIEETEHTEQKRNVIRIIPHHNYNAAINKYNHDIALLELDEPLVLNSYVTPICIADKEYTNIFLKFGSGYVSGWGRVFHKGRSALVLQYLRVPLVDRATCLRSTKFTIYNNMFCAGFHEGGRDSCQGDSGGPHVTEVEGTSFLTGIISWGEECAMKGKYGIYTKVSRYVNWIKEKTKLTSSSSKAPPPSLPSPSRLPGPSDTPILPQSSSSKAPPPSLPSPSRLPGPSDTPILPQSSSSKAPPPSLPSPSRLPGPSDTPILPQ

SEQ ID NO: 114 - protein, 121 aa, Artificial Sequence
  CTP-modified OXM without SP
HSQGTFTSDYSKYLDSRRAQDFVQWLMNTKRNRNNIASSSSKAPPPSLPSPSRLPGPSDTPILPQSSSSKAPPPSLPSPSRLPGPSDTPILPQSSSSKAPPPSLPSPSRLPGPSDTPILPQ

SEQ ID NO: 115 - protein, 26 aa, Artificial Sequence
  SP used for CTP-modified OXM
MATGSRTSLLLAFGLLCLPWLQEGSA